European Patent Specification EP 3 802 677 B1, published April 17, 2024. Title: Mesoporous elastomer. Applicant: Amferia AB. The sequence listing filed with the application follows.

SEQUENCE LISTING (2 sequences)

SEQ ID NO: 1 - protein, 13 aa, Artificial Sequence
  synthetic peptide
  MOD_RES 13: AMIDATION
RRPRPRPWWWWRP

SEQ ID NO: 2 - protein, 13 aa, Artificial Sequence
  syntehtic peptide
  MOD_RES 13: AMIDATION
RRPRPWWRPWWRP